European Patent Application EP 4 151 649 A1, published March 22, 2023. Title: IL-5 BINDING MOLECULE, PREPARATION METHOD THEREFOR, AND USE THEREOF. Applicant: REGENECORE BIOTECH CO., LTD. The sequence listing filed with the application follows.

SEQUENCE LISTING (87 sequences)

SEQ ID NO: 1 - protein, 120 aa, artificial sequence
QVQLVESGGGSVQAGGSLRLSCAASGITASTSCMGWFRQSPGKEREGSLATIYDGSTSYADSVKGRFTISVDNAKNILYLQMNNLKPEDTAMYYCAAAKYCMFWSHPSYWGQGTQVTVSS

SEQ ID NO: 2 - protein, 120 aa, artificial sequence
QVQLVESGGGSVQAGGSLRLSCAASGITASTSCMGWFRQSPGKEREGSLATIYDGSTSYADSVKGQFTISVDNAKNILYLQMNNLKPEDTAMYYCAAAKYCMFWSHPSYWGQGTQVTVSS

SEQ ID NO: 3 - protein, 122 aa, artificial sequence
QVQLVESGGGSAQAGGSLRLSCAASGNTLDLMAWFRQAPGKEREGVAGIYSSGTTYYADSVKGRFTVSRDNAKNTVYLQMNSLKPEDAAMYYCAAKVSWYGRWYQSETYEYWGQGTQVTVSS

SEQ ID NO: 4 - protein, 122 aa, artificial sequence
QVQLVESGGGSVQAGGSLRLSCAASGNTFSFSTYCMGWFRQSPGKEREGSLATIYDGSTAYAGSVKGRFTISVDNAKNILYLQMNNLKPEDTAMYYCAAAKYCMFWSDPSYWGQGTQVTVSS

SEQ ID NO: 5 - protein, 120 aa, artificial sequence
QVQLVESGGGSVQAGGSLRLSCAASGITASTSCMGWFRQSPGKEREGSLATIYDGSTSYADSVKGRFTISVDNAKNILYLQMNNLKPADTAMYYCAAAKYCMFWSHPSYWGQGTQVTVSS

SEQ ID NO: 6 - protein, 120 aa, artificial sequence
QVQLVESGGGSVQAGGSLRLSCAASGITSSTSCMGWFRQSPGKEREGSLATIYDGNISYADSVKGRFTISVDNAKNILYLQMNNLKPEDTAMYYCAAAKYCMFWSDPSYWGQGTQVTVSS

SEQ ID NO: 7 - protein, 122 aa, artificial sequence
QVQLVESGGGSVQAGGSLRLSCVASGLTLNDVSMAWFRQAPGKEREEVAGIDIDGLISYADSVKGRFTISKDNAQNTLYLQMNSLKPEDTAMYSCAAVRLYFSSSRNQYKYEGQGTQVTVSS

SEQ ID NO: 8 - protein, 122 aa, artificial sequence
QVQLVESGGGSVQPGGSLRLSCAASGNTFSFSTYCMGWFRQSPGKEREGSLATIYDGSTAYAGSVKGRFTVSVDNAKNILYLQMNNLKPEDTAMYYCASAKYCMFWSDPSYWGQGTQVTVSS

SEQ ID NO: 9 - protein, 122 aa, artificial sequence
QVQLVESGGGSVQAGGSLRLSCVASGLTLNDVSMAWFRQAPGKEREEVAGIDIDGLISYADPVKGRFTISKDNAQNTMYLQMNSLKPEDTAMYSCAAVRLYFSSSRNQYKYEGQGTQVTVSS

SEQ ID NO: 10 - protein, 122 aa, artificial sequence
QVQLVESGGGSVQAGGSLRLSCAASGNTFSTSTYCMGWFRQSPGKEREGSLATIYDGSTAYAGSVKGRFTISVDNAKNILYLQMNNLKPEDTAMYYCAAAKYCMFWSDPSYWGQGTQVTVSS

SEQ ID NO: 11 - protein, 120 aa, artificial sequence
QVQLVESGGGSVQAGGSLRLSCAASGITSSTSCMGWFRQSPGKEREGSLATIYDGAISYADSVKGRFTISVDNAKNILYLQMNNLKPEDTAMYYCAAAKYCMFWSDPSYWGQGTQVTVSS

SEQ ID NO: 12 - protein, 120 aa, artificial sequence
QVQLVESEGGSVQAGGSLRLSCAVSGITSSTACMGWFRQSPGKEREGSLATIYDGSISYADSVKGRFTISVDNAKNILYLQMNNLKPEDTAMYYCAAAKYCMFWSDPSYWGQGTQVTVSS

SEQ ID NO: 13 - protein, 120 aa, artificial sequence
QVQLVESGGGLVQPGGSLRLSCAASGITASTSCMGWFRQAPGKGLEAVAATIYDGSTYYADSVKGRFTISRDNSKNTLYLQMNSLRAEDTAVYYCAAARYCMFWSHPSYWGQGTLVTVSS

SEQ ID NO: 14 - protein, 120 aa, artificial sequence
QVQLVESGGGSVQAGGSLRLSCAASGITASTSCMGWFRQSPGKEREGSLATIYDASTSYADSVKGRFTISRDNSKNILYLQMNNLRAEDTAVYYCAAARYCMFWSHPSYWGQGTQVTVSS

SEQ ID NO: 15 - protein, 120 aa, artificial sequence
QVQLVESGGGSVQAGGSLRLSCAASGITASTSCMGWFRQSPGKEREGSLATIYDASTSYADSVKGRFTISVDNAKNILYLQMNNLKPEDTAMYYCAAARYCMFWSHPSYWGQGTQVTVSS

SEQ ID NO: 16 - protein, 120 aa, artificial sequence
QVQLVESGGGSVQAGGSLRLSCAASGITASTSCMGWFRQSPGKEREGSLATIYDASTSYADSVKGRFTISRDNAKNILYLQMNNLRAEDTAVYYCAAARYCMFWSHPSYWGQGTQVTVSS

SEQ ID NO: 17 - protein, 120 aa, artificial sequence
QVQLVESGGGSVQAGGSLRLSCAASGITASTSCMGWFRQSPGKEREGSLATIYDGSTSYADSVKGRFTISRDNSKNILYLQMNNLRAEDTAVYYCAAARYCMFWSHPSYWGQGTQVTVSS

SEQ ID NO: 18 - protein, 122 aa, artificial sequence
QVQLVESGGGLVQPGGSLRLSCAASGNTFSFSTYCMGWFRQAPGKGLEAVAATIYDGSTYYAGSVKGRFTISRDNSKNTLYLQMNSLRAEDTAVYYCAAARYCMFWSHPSYWGQGTLVTVSS

SEQ ID NO: 19 - protein, 122 aa, artificial sequence
QVQLVESGGGSVQAGGSLRLSCAASGNTFSFSTYCMGWFRQSPGKEREGSLATIYDASTAYAGSVKGRFTISRDNSKNILYLQMNNLRAEDTAVYYCAAARYCMFWSHPSYWGQGTQVTVSS

SEQ ID NO: 20 - protein, 122 aa, artificial sequence
QVQLVESGGGSVQAGGSLRLSCAASGNTFSFSTYCMGWFRQSPGKEREGSLATIYDASTAYAGSVKGRFTISVDNAKNILYLQMNNLKPEDTAMYYCAAARYCMFWSHPSYWGQGTQVTVSS

SEQ ID NO: 21 - protein, 122 aa, artificial sequence
QVQLVESGGGSVQAGGSLRLSCAASGNTFSFSTYCMGWFRQSPGKEREGSLATIYDASTAYAGSVKGRFTISRDNAKNILYLQMNNLRAEDTAVYYCAAARYCMFWSHPSYWGQGTQVTVSS

SEQ ID NO: 22 - DNA, 360 bp, artificial sequence
caggtgcagctggtggaaagcggcggcggcagcgtgcaggcgggcggcagcctgcgtctgagctgcgcggcgagcggcattaccgcgagcaccagctgcatgggctggtttcgtcagagcccgggcaaagaacgtgaaggcagcctggcgaccatttatgatggcagcaccagctatgcggatagcgtgaaaggccgttttaccattagcgtggataacgcgaaaaacattctgtatctgcagatgaacaacctgaaaccggaagataccgcgatgtattattgcgcggcggcgaaatattgcatgttttggagccatccgagctattggggccagggcacccaggtgaccgtgagcagc

SEQ ID NO: 23 - DNA, 360 bp, artificial sequence
caggtgcagctggtggaaagcggcggcggcagcgtgcaggcgggcggcagcctgcgtctgagctgcgcggcgagcggcattaccgcgagcaccagctgcatgggctggtttcgtcagagcccgggcaaagaacgtgaaggcagcctggcgaccatttatgatggcagcaccagctatgcggatagcgtgaaaggccagtttaccattagcgtggataacgcgaaaaacattctgtatctgcagatgaacaacctgaaaccggaagataccgcgatgtattattgcgcggcggcgaaatattgcatgttttggagccatccgagctattggggccagggcacccaggtgaccgtgagcagc

SEQ ID NO: 24 - DNA, 366 bp, artificial sequence
caggtgcagctggtggaaagcggcggcggcagcgcgcaggcgggcggcagcctgcgtctgagctgcgcggcgagcggcaacaccctggatctgatggcgtggtttcgtcaggcgccgggcaaagaacgtgaaggcgtggcgggcatttatagcagcggcaccacctattatgcggatagcgtgaaaggccgttttaccgtgagccgtgataacgcgaaaaacaccgtgtatctgcagatgaacagcctgaaaccggaagatgcggcgatgtattattgcgcggcgaaagtgagctggtatggccgttggtatcagagcgaaacctatgaatattggggccagggcacccaggtgaccgtgagcagc

SEQ ID NO: 25 - DNA, 366 bp, artificial sequence
caggtgcagctggtggaaagcggcggcggcagcgtgcaggcgggcggcagcctgcgtctgagctgcgcggcgagcggcaacacctttagctttagcacctattgcatgggctggtttcgtcagagcccgggcaaagaacgtgaaggcagcctggcgaccatttatgatggcagcaccgcgtatgcgggcagcgtgaaaggccgttttaccattagcgtggataacgcgaaaaacattctgtatctgcagatgaacaacctgaaaccggaagataccgcgatgtattattgcgcggcggcgaaatattgcatgttttggagcgatccgagctattggggccagggcacccaggtgaccgtgagcagc

SEQ ID NO: 26 - DNA, 360 bp, artificial sequence
caggtgcagctggtggaaagcggcggcggcagcgtgcaggcgggcggcagcctgcgtctgagctgcgcggcgagcggcattaccgcgagcaccagctgcatgggctggtttcgtcagagcccgggcaaagaacgtgaaggcagcctggcgaccatttatgatggcagcaccagctatgcggatagcgtgaaaggccgttttaccattagcgtggataacgcgaaaaacattctgtatctgcagatgaacaacctgaaaccggcggataccgcgatgtattattgcgcggcggcgaaatattgcatgttttggagccatccgagctattggggccagggcacccaggtgaccgtgagcagc

SEQ ID NO: 27 - DNA, 360 bp, artificial sequence
caggtgcagctggtggaaagcggcggcggcagcgtgcaggcgggcggcagcctgcgtctgagctgcgcggcgagcggcattaccagcagcaccagctgcatgggctggtttcgtcagagcccgggcaaagaacgtgaaggcagcctggcgaccatttatgatggcaacattagctatgcggatagcgtgaaaggccgttttaccattagcgtggataacgcgaaaaacattctgtatctgcagatgaacaacctgaaaccggaagataccgcgatgtattattgcgcggcggcgaaatattgcatgttttggagcgatccgagctattggggccagggcacccaggtgaccgtgagcagc

SEQ ID NO: 28 - DNA, 366 bp, artificial sequence
caggtgcagctggtggaaagcggcggcggcagcgtgcaggcgggcggcagcctgcgtctgagctgcgtggcgagcggcctgaccctgaacgatgtgagcatggcgtggtttcgtcaggcgccgggcaaagaacgtgaagaagtggcgggcattgatattgatggcctgattagctatgcggatagcgtgaaaggccgttttaccattagcaaagataacgcgcagaacaccctgtatctgcagatgaacagcctgaaaccggaagataccgcgatgtatagctgcgcggcggtgcgtctgtattttagcagcagccgtaaccagtataaatatgaaggccagggcacccaggtgaccgtgagcagc

SEQ ID NO: 29 - DNA, 366 bp, artificial sequence
caggtgcagctggtggaaagcggcggcggcagcgtgcagccgggcggcagcctgcgtctgagctgcgcggcgagcggcaacacctttagctttagcacctattgcatgggctggtttcgtcagagcccgggcaaagaacgtgaaggcagcctggcgaccatttatgatggcagcaccgcgtatgcgggcagcgtgaaaggccgttttaccgtgagcgtggataacgcgaaaaacattctgtatctgcagatgaacaacctgaaaccggaagataccgcgatgtattattgcgcgagcgcgaaatattgcatgttttggagcgatccgagctattggggccagggcacccaggtgaccgtgagcagc

SEQ ID NO: 30 - DNA, 366 bp, artificial sequence
caggtgcagctggtggaaagcggcggcggcagcgtgcaggcgggcggcagcctgcgtctgagctgcgtggcgagcggcctgaccctgaacgatgtgagcatggcgtggtttcgtcaggcgccgggcaaagaacgtgaagaagtggcgggcattgatattgatggcctgattagctatgcggatccggtgaaaggccgttttaccattagcaaagataacgcgcagaacaccatgtatctgcagatgaacagcctgaaaccggaagataccgcgatgtatagctgcgcggcggtgcgtctgtattttagcagcagccgtaaccagtataaatatgaaggccagggcacccaggtgaccgtgagcagc

SEQ ID NO: 31 - DNA, 366 bp, artificial sequence
caggtgcagctggtggaaagcggcggcggcagcgtgcaggcgggcggcagcctgcgtctgagctgcgcggcgagcggcaacacctttagcaccagcacctattgcatgggctggtttcgtcagagcccgggcaaagaacgtgaaggcagcctggcgaccatttatgatggcagcaccgcgtatgcgggcagcgtgaaaggccgttttaccattagcgtggataacgcgaaaaacattctgtatctgcagatgaacaacctgaaaccggaagataccgcgatgtattattgcgcggcggcgaaatattgcatgttttggagcgatccgagctattggggccagggcacccaggtgaccgtgagcagc

SEQ ID NO: 32 - DNA, 360 bp, artificial sequence
caggtgcagctggtggaaagcggcggcggcagcgtgcaggcgggcggcagcctgcgtctgagctgcgcggcgagcggcattaccagcagcaccagctgcatgggctggtttcgtcagagcccgggcaaagaacgtgaaggcagcctggcgaccatttatgatggcgcgattagctatgcggatagcgtgaaaggccgttttaccattagcgtggataacgcgaaaaacattctgtatctgcagatgaacaacctgaaaccggaagataccgcgatgtattattgcgcggcggcgaaatattgcatgttttggagcgatccgagctattggggccagggcacccaggtgaccgtgagcagc

SEQ ID NO: 33 - DNA, 360 bp, artificial sequence
caggtgcagctggtggaaagcgaaggcggcagcgtgcaggcgggcggcagcctgcgtctgagctgcgcggtgagcggcattaccagcagcaccgcgtgcatgggctggtttcgtcagagcccgggcaaagaacgtgaaggcagcctggcgaccatttatgatggcagcattagctatgcggatagcgtgaaaggccgttttaccattagcgtggataacgcgaaaaacattctgtatctgcagatgaacaacctgaaaccggaagataccgcgatgtattattgcgcggcggcgaaatattgcatgttttggagcgatccgagctattggggccagggcacccaggtgaccgtgagcagc

SEQ ID NO: 34 - DNA, 360 bp, artificial sequence
caggtgcagctggtggaaagcggcggcggcctggtgcagccgggcggcagcctgcgtctgagctgcgcggcgagcggcattaccgcgagcaccagctgcatgggctggtttcgtcaggcgccgggcaaaggcctggaagcggtggcggcgaccatttatgatggcagcacctattatgcggatagcgtgaaaggccgttttaccattagccgtgataacagcaaaaacaccctgtatctgcagatgaacagcctgcgtgcggaagataccgcggtgtattattgcgcggcggcgcgttattgcatgttttggagccatccgagctattggggccagggcaccctggtgaccgtgagcagc

SEQ ID NO: 35 - DNA, 360 bp, artificial sequence
caggtgcagctggtggaaagcggcggcggcagcgtgcaggcgggcggcagcctgcgtctgagctgcgcggcgagcggcattaccgcgagcaccagctgcatgggctggtttcgtcagagcccgggcaaagaacgtgaaggcagcctggcgaccatttatgatgcgagcaccagctatgcggatagcgtgaaaggccgttttaccattagccgtgataacagcaaaaacattctgtatctgcagatgaacaacctgcgtgcggaagataccgcggtgtattattgcgcggcggcgcgttattgcatgttttggagccatccgagctattggggccagggcacccaggtgaccgtgagcagc

SEQ ID NO: 36 - DNA, 360 bp, artificial sequence
caggtgcagctggtggaaagcggcggcggcagcgtgcaggcgggcggcagcctgcgtctgagctgcgcggcgagcggcattaccgcgagcaccagctgcatgggctggtttcgtcagagcccgggcaaagaacgtgaaggcagcctggcgaccatttatgatgcgagcaccagctatgcggatagcgtgaaaggccgttttaccattagcgtggataacgcgaaaaacattctgtatctgcagatgaacaacctgaaaccggaagataccgcgatgtattattgcgcggcggcgcgttattgcatgttttggagccatccgagctattggggccagggcacccaggtgaccgtgagcagc

SEQ ID NO: 37 - DNA, 360 bp, artificial sequence
caggtgcagctggtggaaagcggcggcggcagcgtgcaggcgggcggcagcctgcgtctgagctgcgcggcgagcggcattaccgcgagcaccagctgcatgggctggtttcgtcagagcccgggcaaagaacgtgaaggcagcctggcgaccatttatgatgcgagcaccagctatgcggatagcgtgaaaggccgttttaccattagccgtgataacgcgaaaaacattctgtatctgcagatgaacaacctgcgtgcggaagataccgcggtgtattattgcgcggcggcgcgttattgcatgttttggagccatccgagctattggggccagggcacccaggtgaccgtgagcagc

SEQ ID NO: 38 - DNA, 360 bp, artificial sequence
caggtgcagctggtggaaagcggcggcggcagcgtgcaggcgggcggcagcctgcgtctgagctgcgcggcgagcggcattaccgcgagcaccagctgcatgggctggtttcgtcagagcccgggcaaagaacgtgaaggcagcctggcgaccatttatgatggcagcaccagctatgcggatagcgtgaaaggccgttttaccattagccgtgataacagcaaaaacattctgtatctgcagatgaacaacctgcgtgcggaagataccgcggtgtattattgcgcggcggcgcgttattgcatgttttggagccatccgagctattggggccagggcacccaggtgaccgtgagcagc

SEQ ID NO: 39 - DNA, 366 bp, artificial sequence
caggtgcagctggtggaaagcggcggcggcctggtgcagccgggcggcagcctgcgtctgagctgcgcggcgagcggcaacacctttagctttagcacctattgcatgggctggtttcgtcaggcgccgggcaaaggcctggaagcggtggcggcgaccatttatgatggcagcacctattatgcgggcagcgtgaaaggccgttttaccattagccgtgataacagcaaaaacaccctgtatctgcagatgaacagcctgcgtgcggaagataccgcggtgtattattgcgcggcggcgcgttattgcatgttttggagccatccgagctattggggccagggcaccctggtgaccgtgagcagc

SEQ ID NO: 40 - DNA, 366 bp, artificial sequence
caggtgcagctggtggaaagcggcggcggcagcgtgcaggcgggcggcagcctgcgtctgagctgcgcggcgagcggcaacacctttagctttagcacctattgcatgggctggtttcgtcagagcccgggcaaagaacgtgaaggcagcctggcgaccatttatgatgcgagcaccgcgtatgcgggcagcgtgaaaggccgttttaccattagccgtgataacagcaaaaacattctgtatctgcagatgaacaacctgcgtgcggaagataccgcggtgtattattgcgcggcggcgcgttattgcatgttttggagccatccgagctattggggccagggcacccaggtgaccgtgagcagc

SEQ ID NO: 41 - DNA, 366 bp, artificial sequence
caggtgcagctggtggaaagcggcggcggcagcgtgcaggcgggcggcagcctgcgtctgagctgcgcggcgagcggcaacacctttagctttagcacctattgcatgggctggtttcgtcagagcccgggcaaagaacgtgaaggcagcctggcgaccatttatgatgcgagcaccgcgtatgcgggcagcgtgaaaggccgttttaccattagcgtggataacgcgaaaaacattctgtatctgcagatgaacaacctgaaaccggaagataccgcgatgtattattgcgcggcggcgcgttattgcatgttttggagccatccgagctattggggccagggcacccaggtgaccgtgagcagc

SEQ ID NO: 42 - DNA, 366 bp, artificial sequence
caggtgcagctggtggaaagcggcggcggcagcgtgcaggcgggcggcagcctgcgtctgagctgcgcggcgagcggcaacacctttagctttagcacctattgcatgggctggtttcgtcagagcccgggcaaagaacgtgaaggcagcctggcgaccatttatgatgcgagcaccgcgtatgcgggcagcgtgaaaggccgttttaccattagccgtgataacgcgaaaaacattctgtatctgcagatgaacaacctgcgtgcggaagataccgcggtgtattattgcgcggcggcgcgttattgcatgttttggagccatccgagctattggggccagggcacccaggtgaccgtgagcagc

SEQ ID NO: 43 - protein, 8 aa, artificial sequence
GITASTSC

SEQ ID NO: 44 - protein, 8 aa, artificial sequence
GITSSTAC

SEQ ID NO: 45 - protein, 8 aa, artificial sequence
GITSSTSC

SEQ ID NO: 46 - protein, 8 aa, artificial sequence
GLTLNDVS

SEQ ID NO: 47 - protein, 10 aa, artificial sequence
GNTFSFSTYC

SEQ ID NO: 48 - protein, 10 aa, artificial sequence
GNTFSTSTYC

SEQ ID NO: 49 - protein, 6 aa, artificial sequence
GNTLDL

SEQ ID NO: 50 - protein, 7 aa, artificial sequence
IDIDGLI

SEQ ID NO: 51 - protein, 7 aa, artificial sequence
IYSSGTT

SEQ ID NO: 52 - protein, 7 aa, artificial sequence
TIYDAST

SEQ ID NO: 53 - protein, 7 aa, artificial sequence
TIYDGAI

SEQ ID NO: 54 - protein, 7 aa, artificial sequence
TIYDGNI

SEQ ID NO: 55 - protein, 7 aa, artificial sequence
TIYDGSI

SEQ ID NO: 56 - protein, 7 aa, artificial sequence
TIYDGST

SEQ ID NO: 57 - protein, 15 aa, artificial sequence
AAAKYCMFWSDPSYW

SEQ ID NO: 58 - protein, 15 aa, artificial sequence
AAAKYCMFWSHPSYW

SEQ ID NO: 59 - protein, 15 aa, artificial sequence
AAARYCMFWSHPSYW

SEQ ID NO: 60 - protein, 19 aa, artificial sequence
AAKVSWYGRWYQSETYEYW

SEQ ID NO: 61 - protein, 17 aa, artificial sequence
AAVRLYFSSSRNQYKYE

SEQ ID NO: 62 - protein, 15 aa, artificial sequence
ASAKYCMFWSDPSYW

SEQ ID NO: 63 - protein, 25 aa, artificial sequence
QVQLVESEGGSVQAGGSLRLSCAVS

SEQ ID NO: 64 - protein, 25 aa, artificial sequence
QVQLVESGGGSAQAGGSLRLSCAAS

SEQ ID NO: 65 - protein, 25 aa, artificial sequence
QVQLVESGGGSVQAGGSLRLSCAAS

SEQ ID NO: 66 - protein, 25 aa, artificial sequence
QVQLVESGGGSVQAGGSLRLSCVAS

SEQ ID NO: 67 - protein, 25 aa, artificial sequence
QVQLVESGGGLVQPGGSLRLSCAAS

SEQ ID NO: 68 - protein, 25 aa, artificial sequence
QVQLVESGGGSVQPGGSLRLSCAAS

SEQ ID NO: 69 - protein, 17 aa, artificial sequence
MAWFRQAPGKEREEVAG

SEQ ID NO: 70 - protein, 17 aa, artificial sequence
MGWFRQAPGKGLEAVAA

SEQ ID NO: 71 - protein, 17 aa, artificial sequence
MAWFRQAPGKEREGVAG

SEQ ID NO: 72 - protein, 17 aa, artificial sequence
MGWFRQSPGKEREGSLA

SEQ ID NO: 73 - protein, 38 aa, artificial sequence
AYAGSVKGRFTISVDNAKNILYLQMNNLKPEDTAMYYC

SEQ ID NO: 74 - protein, 38 aa, artificial sequence
AYAGSVKGRFTISRDNSKNILYLQMNNLRAEDTAVYYC

SEQ ID NO: 75 - protein, 38 aa, artificial sequence
AYAGSVKGRFTISRDNAKNILYLQMNNLRAEDTAVYYC

SEQ ID NO: 76 - protein, 38 aa, artificial sequence
AYAGSVKGRFTVSVDNAKNILYLQMNNLKPEDTAMYYC

SEQ ID NO: 77 - protein, 38 aa, artificial sequence
SYADSVKGRFTISRDNAKNILYLQMNNLRAEDTAVYYC

SEQ ID NO: 78 - protein, 38 aa, artificial sequence
SYADSVKGRFTISRDNSKNILYLQMNNLRAEDTAVYYC

SEQ ID NO: 79 - protein, 38 aa, artificial sequence
SYADPVKGRFTISKDNAQNTMYLQMNSLKPEDTAMYSC

SEQ ID NO: 80 - protein, 38 aa, artificial sequence
YYADSVKGRFTISRDNSKNTLYLQMNSLRAEDTAVYYC

SEQ ID NO: 81 - protein, 38 aa, artificial sequence
YYAGSVKGRFTISRDNSKNTLYLQMNSLRAEDTAVYYC

SEQ ID NO: 82 - protein, 38 aa, artificial sequence
SYADSVKGQFTISVDNAKNILYLQMNNLKPEDTAMYYC

SEQ ID NO: 83 - protein, 38 aa, artificial sequence
SYADSVKGRFTISKDNAQNTLYLQMNSLKPEDTAMYSC

SEQ ID NO: 84 - protein, 38 aa, artificial sequence
SYADSVKGRFTISVDNAKNILYLQMNNLKPADTAMYYC

SEQ ID NO: 85 - protein, 38 aa, artificial sequence
SYADSVKGRFTISVDNAKNILYLQMNNLKPEDTAMYYC

SEQ ID NO: 86 - protein, 38 aa, artificial sequence
YYADSVKGRFTVSRDNAKNTVYLQMNSLKPEDAAMYYC

SEQ ID NO: 87 - protein, 10 aa, artificial sequence
GQGTQVTVSS